European Patent Application EP 4 375 293 A1, published May 29, 2024. Title: VHH antibodies against SARS-CoV-2 Omicron variants. Applicant: Max-Planck Gesellschaft zur Förderung der Wissenschaften e.V. The sequence listing filed with the application follows.

SEQUENCE LISTING (31 sequences)

SEQ ID NO: 1 - protein, 130 aa, synthetic construct
QVQLVESGGGLVQPGGSLRLSCVVSELGLDYYQIGWFRQAPGKEREGVSCFRSSDEIRYYADSVKGRFTTFRDNAGTTVYLQMNSLKPEDTGVYYCAVAPQTYYHGTWYGECAAAGMDSWGKGTQVTVSS

SEQ ID NO: 2 - protein, 9 aa, synthetic construct
LGLDYYQIG

SEQ ID NO: 3 - protein, 15 aa, synthetic construct
SCFRSSDEIRYYADS

SEQ ID NO: 4 - protein, 22 aa, synthetic construct
VAPQTYYHGTWYGECAAAGMDS

SEQ ID NO: 5 - protein, 130 aa, synthetic construct
QVQLVESGGGLVQPGGSLRLSCVVSDLGLDYYQIGWFRQAPGKEREGVSCFRSSDEIRYYADPVKGRFTTFRDNAGTTVYLQMNSLKPEDTGVYYCAVAPQTYYHGTWYGECAAAGMDSWGKGTLVTVSS

SEQ ID NO: 6 - protein, 15 aa, synthetic construct
SCFRSSDEIRYYADP

SEQ ID NO: 7 - protein, 127 aa, synthetic construct
QVQLVESGGGLVQPGGSLRLSCATSGLTLDHYAIGWFLQAPGKEREGVACVSDDERSLYAPSVMGRFSISRDNAKKTFYLEMNSLKPEDTGVYYCASGPVVPGTLCRIPTVLGYDDWGQGTQVTVSS

SEQ ID NO: 8 - protein, 9 aa, synthetic construct
LTLDHYAIG

SEQ ID NO: 9 - protein, 14 aa, synthetic construct
ACVSDDERSLYAPS

SEQ ID NO: 10 - protein, 20 aa, synthetic construct
SGPVVPGTLCRIPTVLGYDD

SEQ ID NO: 11 - protein, 128 aa, synthetic construct
QVQLVESGGGLVQPGGSLRLSCATSEIGLSYYGVGWFLQAPGKDREGVACMHNTDGNPVYAPSVKGRFTISRDDAKKMVYLEMNNLKPEDTGVYYCAVGPLSPGITCRIPTTLGYDDWGQGTQVTVSS

SEQ ID NO: 12 - protein, 9 aa, synthetic construct
IGLSYYGVG

SEQ ID NO: 13 - protein, 15 aa, synthetic construct
ACMHNTDGNPVYAPS

SEQ ID NO: 14 - protein, 20 aa, synthetic construct
VGPLSPGITCRIPTTLGYDD

SEQ ID NO: 15 - protein, 116 aa, synthetic construct
QVQLVESGGGLVRTGGSLRLSCAASGSILQIWAMKWYRQAPGLQREWIATIPNSGEPFYASSVEGRFTGSRENEETVYLYLNNLEPEDTAVYYCEVNEGVPVREYWGQGTQVTVSS

SEQ ID NO: 16 - protein, 9 aa, synthetic construct
SILQIWAMK

SEQ ID NO: 17 - protein, 14 aa, synthetic construct
ATIPNSGEPFYASS

SEQ ID NO: 18 - protein, 10 aa, synthetic construct
VNEGVPVREY

SEQ ID NO: 19 - protein, 130 aa, synthetic construct
QVQLVESGGGLVQPGGSLRLSCAASGFTLDYYAIGWFRQAPGKEREGVSRISSSDGSTDYADSVKGRFTISRDNAKNTVYLQMNSLKPEDTAVYYCATVPGTYYSGNWYYTWHPKAVDYWGKGTLVTVSS

SEQ ID NO: 20 - protein, 9 aa, synthetic construct
FTLDYYAIG

SEQ ID NO: 21 - protein, 15 aa, synthetic construct
SRISSSDGSTDYADS

SEQ ID NO: 22 - protein, 22 aa, synthetic construct
TVPGTYYSGNWYYTWHPKAVDY

SEQ ID NO: 23 - protein, 231 aa, unidentified
ETNLCPFGEVFNATRFASVYAWNRKRISNCVADYSVLYNSASFSTFKCYGVSPTKLNDLCFTNVYADSFVIRGDEVRQIAPGQTGKIADYNYKLPDDFTGCVIAWNSNNLDSKVGGNYNYLYRLFRKSNLKPFERDISTEIYQAGSTPCNGVEGFNCYFPLQSYGFQPTNGVGYQPYRVVVLSFELLHAPATVCGPKTGTGGSGGSGLNDIFEAQKIEWHEGRTKHHHHHH

SEQ ID NO: 24 - protein, 231 aa, unidentified
ETNLCPFGEVFNATRFASVYAWNRKRISNCVADYSVLYNSASFSTFKCYGVSPTKLNDLCFTNVYADSFVIRGDEVRQIAPGQTGKIADYNYKLPDDFTGCVIAWNSNNLDSKVGGNYNYRYRLFRKSNLKPFERDISTEIYQAGSKPCNGVEGFNCYFPLQSYGFQPTNGVGYQPYRVVVLSFELLHAPATVCGPKTGTGGSGGSGLNDIFEAQKIEWHEGRTKHHHHHH

SEQ ID NO: 25 - protein, 248 aa, unidentified
ETGNLCPFDEVFNATRFASVYAWNRKRISNCVADYSVLYNLAPFFTFKCYGVSPTKLNDLCFTNVYADSFVIRGDEVRQIAPGQTGNIADYNYKLPDDFTGCVIAWNSNKLDSKVSGNYNYLYRLFRKSNLKPFERDISTEIYQAGNKPCNGVAGFNCYFPLRSYSFRPTYGVGHQPYRVVVLSFELLHAPATVCGPKGTGGSGGSGLNDIFEAQKIEWHEGGSGRSHHHHSGHHHTGHHHHSGSHHH

SEQ ID NO: 26 - protein, 248 aa, unidentified
ETGNLCPFDEVFNATRFASVYAWNRKRISNCVADYSVLYNFAPFFAFKCYGVSPTKLNDLCFTNVYADSFVIRGNEVSQIAPGQTGNIADYNYKLPDDFTGCVIAWNSNKLDSKVGGNYNYRYRLFRKSNLKPFERDISTEIYQAGNKPCNGVAGVNCYFPLQSYGFRPTYGVGHQPYRVVVLSFELLHAPATVCGPKGTGGSGGSGLNDIFEAQKIEWHEGGSGRSHHHHSGHHHTGHHHHSGSHHH

SEQ ID NO: 27 - protein, 248 aa, unidentified
ETGNLCPFHEVFNATRFASVYAWNRKRISNCVADYSVLYNFAPFFAFKCYGVSPTKLNDLCFTNVYADSFVIRGNEVSQIAPGQTGNIADYNYKLPDDFTGCVIAWNSNKLDSKVSGNYNYLYRLFRKSKLKPFERDISTEIYQAGNKPCNGVAGFNCYFPLQSYGFRPTYGVGHQPYRVVVLSFELLHAPATVCGPKGTGGSGGSGLNDIFEAQKIEWHEGGSGRSHHHHSGHHHTGHHHHSGSHHH

SEQ ID NO: 28 - protein, 14 aa, synthetic construct
SCFRSSDEIRYYAD

SEQ ID NO: 29 - protein, 15 aa, synthetic construct
  VARIANT 15: note = X can be any natural amino acid
SCFRSSDEIRYYADX

SEQ ID NO: 30 - protein, 130 aa, synthetic construct
  VARIANT 26: note = X is D or E
  VARIANT 63: note = X is P or S
  VARIANT 125: note = X is L or Q
QVQLVESGGGLVQPGGSLRLSCVVSXLGLDYYQIGWFRQAPGKEREGVSCFRSSDEIRYYADXVKGRFTTFRDNAGTTVYLQMNSLKPEDTGVYYCAVAPQTYYHGTWYGECAAAGMDSWGKGTXVTVSS

SEQ ID NO: 31 - protein, 1273 aa, unidentified
MFVFLVLLPLVSSQCVNLTTRTQLPPAYTNSFTRGVYYPDKVFRSSVLHSTQDLFLPFFSNVTWFHAIHVSGTNGTKRFDNPVLPFNDGVYFASTEKSNIIRGWIFGTTLDSKTQSLLIVNNATNVVIKVCEFQFCNDPFLGVYYHKNNKSWMESEFRVYSSANNCTFEYVSQPFLMDLEGKQGNFKNLREFVFKNIDGYFKIYSKHTPINLVRDLPQGFSALEPLVDLPIGINITRFQTLLALHRSYLTPGDSSSGWTAGAAAYYVGYLQPRTFLLKYNENGTITDAVDCALDPLSETKCTLKSFTVEKGIYQTSNFRVQPTESIVRFPNITNLCPFGEVFNATRFASVYAWNRKRISNCVADYSVLYNSASFSTFKCYGVSPTKLNDLCFTNVYADSFVIRGDEVRQIAPGQTGKIADYNYKLPDDFTGCVIAWNSNNLDSKVGGNYNYLYRLFRKSNLKPFERDISTEIYQAGSTPCNGVEGFNCYFPLQSYGFQPTNGVGYQPYRVVVLSFELLHAPATVCGPKKSTNLVKNKCVNFNFNGLTGTGVLTESNKKFLPFQQFGRDIADTTDAVRDPQTLEILDITPCSFGGVSVITPGTNTSNQVAVLYQDVNCTEVPVAIHADQLTPTWRVYSTGSNVFQTRAGCLIGAEHVNNSYECDIPIGAGICASYQTQTNSPRRARSVASQSIIAYTMSLGAENSVAYSNNSIAIPTNFTISVTTEILPVSMTKTSVDCTMYICGDSTECSNLLLQYGSFCTQLNRALTGIAVEQDKNTQEVFAQVKQIYKTPPIKDFGGFNFSQILPDPSKPSKRSFIEDLLFNKVTLADAGFIKQYGDCLGDIAARDLICAQKFNGLTVLPPLLTDEMIAQYTSALLAGTITSGWTFGAGAALQIPFAMQMAYRFNGIGVTQNVLYENQKLIANQFNSAIGKIQDSLSSTASALGKLQDVVNQNAQALNTLVKQLSSNFGAISSVLNDILSRLDKVEAEVQIDRLITGRLQSLQTYVTQQLIRAAEIRASANLAATKMSECVLGQSKRVDFCGKGYHLMSFPQSAPHGVVFLHVTYVPAQEKNFTTAPAICHDGKAHFPREGVFVSNGTHWFVTQRNFYEPQIITTDNTFVSGNCDVVIGIVNNTVYDPLQPELDSFKEELDKYFKNHTSPDVDLGDISGINASVVNIQKEIDRLNEVAKNLNESLIDLQELGKYEQYIKWPWYIWLGFIAGLIAIVMVTIMLCCMTSCCSCLKGCCSCGSCCKFDEDDSEPVLKGVKLHYT